European Patent Application EP 4 279 503 A1, published November 22, 2023. Title: METHOD AND KIT FOR DETERMINING THE DEGREE OF ENTEROBACTERIAL CONTAMINATION OF FOOD AND BEVERAGE SAMPLE OR ENVIRONMENTAL SAMPLE. Applicant: ASAHI KASEI KABUSHIKI KAISHA. The sequence listing filed with the application follows.

SEQUENCE LISTING (10 sequences)

SEQ ID NO: 1 - protein, 116 aa, Artificial Sequence
  EC50C1 VH
QVQLQQSGAELAKPGASVKMSCKASGYTFTSYWMNWVKQRPGQGLEWIGYINPNTGYTEYDQKFKDKATLTADKSSSTAYMQLSSLTSEDSAVYYCARYWAYFEYWGQGTTLTVSS

SEQ ID NO: 2 - protein, 106 aa, Artificial Sequence
  EC50C1 VL
DIKMTQSPSSMYASLGERVTITCKASQDINSYLSWFQQKPGKSPKTLIYRANRLVDGVPSRFSGSGSGQDYSLTISSLEYEDMGIYYCLQYDEFRTFGGGTKLEIK

SEQ ID NO: 3 - protein, 118 aa, Artificial Sequence
  EC149C3 VH
QVQLQQSGAELVKPGASVKLSCKASDYTFTNFYIYWVKQRPGQGLEWIGEINPSNGYTTFNVKFKSKATLTVDKSSSTAYMQLSSLTSEDSAVYYCTRNYGGSRCAYWGQGTLVTVSA

SEQ ID NO: 4 - protein, 112 aa, Artificial Sequence
  EC149C3 VL
DVLMTQTPLSLPVSLGDQASISCRSSQSIVHSNGNTYLEWYLQKPGQSPKLLIYKVSNRFSGVPDRFSGSGSGTDFTLKISRVEAEDLGVYYCFQGSHVPWTFGGGTKLEIK

SEQ ID NO: 5 - protein, 116 aa, Artificial Sequence
  EC162A3 VH
QVQLQQSGTELAKPGASVQMSCKASGYTFTSYWMHWVKQRPGQGLEWIGYINPNTGYTEYNQQFKDKATLTADKSSSTAYMQLSSLTSEDSAVYYCANYFAWFGYWGQGTLVTVSA

SEQ ID NO: 6 - protein, 107 aa, Artificial Sequence
  EC162A3 VL
DIKMTQSPSSMYASLGERVTVTCKASQDIYSYLNWFQQKPGKSPKTLIYRANRLVDGVPSRFSGSGSGQEYSLTISSLEHEDMGIYYCLQHDQHPYTFGSGTKLEIK

SEQ ID NO: 7 - protein, 118 aa, Artificial Sequence
  PA51B2 VH
QVQLQQPGSVLVRPGASVKLSCKPSGYTFTGSWMHWTKQRPGQGLEWIGEIHPYSGNTNYNEKFRVKATLTVDTSSSTTYVDLSSLTSDDSAVYYCASGDFDAGFTYWGQGTLVTVSA

SEQ ID NO: 8 - protein, 111 aa, Artificial Sequence
  PA51B2 VL
DIVLTQSPASLAVSLGRRATISCKASQSVDYDGDSYMNWYQQKPGQPPKLLIYVASNLESGIPARFSGSGSGTDFTLNIHPVEEEDAATYYCQQTNEDPFTFGAGTKLELK

SEQ ID NO: 9 - protein, 118 aa, Artificial Sequence
  CP141A190.1 VH
QVQLQQPGAELVKPGASVKLSCKTSGYNFTSNWIHWVKQRPGQGLEWIGEINPSNGRANYNEKFKNKATLTVDKSSSTAFMHLSSLTSEDSAVYFCSRGDFDEGFTYWGQGTLVTVSA

SEQ ID NO: 10 - protein, 108 aa, Artificial Sequence
  CP141A190.1 VL
QIVLTQSPAIMSASLGERVTMTCTASSNVNSDYLHWYQQKPGSSPRLWIYTTSNLASGVPTRFSGNGSGTSYSLTISSMEAEDAATYYCHQYHRSPRTFGGGTKLEIK